European Patent Specification EP 3 752 522 B1, published March 27, 2024. Title: NANOPORE PROTEIN CONJUGATES FOR DETECTION AND ANALYSIS OF ANALYTES. Applicant: F. HOFFMANN-LA ROCHE AG ROCHE DIAGNOSTICS GMBH ROCHE DIAGNOSTICS OPERATIONS, INC. The sequence listing filed with the application follows.

SEQUENCE LISTING (17 sequences)

SEQ ID NO: 1 - DNA, 1023 bp, Staphylococcus aureus
atggcagatctcgatcccgcgaaattaatacgactcactatagggaggccacaacggtttccctctagaaataattttgtttaactttaagaaggagatatacaaatggattcagatattaatattaaaacaggtacaacagatattggttcaaatacaacagtaaaaactggtgatttagtaacttatgataaagaaaatggtatgcataaaaaagtattttattcttttattgatgataaaaatcataataaaaaattgttagttattcgtacaaaaggtactattgcaggtcaatatagagtatatagtgaagaaggtgctaataaaagtggtttagcatggccatctgcttttaaagttcaattacaattacctgataatgaagtagcacaaatttcagattattatccacgtaatagtattgatacaaaagaatatatgtcaacattaacttatggttttaatggtaatgtaacaggtgatgatactggtaaaattggtggtttaattggtgctaatgtttcaattggtcatacattaaaatatgtacaaccagattttaaaacaattttagaaagtcctactgataaaaaagttggttggaaagtaatttttaataatatggttaatcaaaattggggtccttatgatcgtgatagttggaatcctgtatatggtaatcaattatttatgaaaacaagaaatggttctatgaaagcagctgataatttcttagatccaaataaagcatcaagtttattatcttcaggtttttctcctgattttgcaacagttattactatggatagaaaagcatcaaaacaacaaacaaatattgatgttatttatgaacgtgtaagagatgattatcaattacattggacatcaactaattggaaaggtacaaatactaaagataaatggacagatagaagttcagaaagatataaaattgattgggaaaaagaagaaatgacaaatggtctcagcgcttggagccacccgcagttcgaaaaataa

SEQ ID NO: 2 - protein, 306 aa, Artificial Sequence
  source: /note="Description of Artificial Sequence: Synthetic polypeptide"
MADSDINIKTGTTDIGSNTTVKTGDLVTYDKENGMHKKVFYSFIDDKNHNKKLLVIRTKGTIAGQYRVYSEEGANKSGLAWPSAFKVQLQLPDNEVAQISDYYPRNSIDTKEYMSTLTYGFNGNVTGDDTGKIGGLIGANVSIGHTLKYVQPDFKTILESPTDKKVGWKVIFNNMVNQNWGPYDRDSWNPVYGNQLFMKTRNGSMKAADNFLDPNKASSLLSSGFSPDFATVITMDRKASKQQTNIDVIYERVRDDYQLHWTSTNWKGTNTKDKWTDRSSERYKIDWEKEEMTNGLSAWSHPQFEK

SEQ ID NO: 3 - protein, 305 aa, Artificial Sequence
  source: /note="Description of Artificial Sequence: Synthetic polypeptide"
ADSDINIKTGTTDIGSNTTVKTGDLVTYDKENGMHKKVFYSFIDDKNHNKKLLVIRTKGTIAGQYRVYSEEGANKSGLAWPSAFKVQLQLPDNEVAQISDYYPRNSIDTKEYMSTLTYGFNGNVTGDDTGKIGGLIGANVSIGHTLKYVQPDFKTILESPTDKKVGWKVIFNNMVNQNWGPYDRDSWNPVYGNQLFMKTRNGSMKAADNFLDPNKASSLLSSGFSPDFATVITMDRKASKQQTNIDVIYERVRDDYQLHWTSTNWKGTNTKDKWTDRSSERYKIDWEKEEMTNGLSAWSHPQFEK

SEQ ID NO: 4 - protein, 381 aa, Artificial Sequence
  source: /note="Description of Artificial Sequence: Synthetic polypeptide"
ADSDINIKTGTTDIGSNTTVKTGDLVTYDKENGMGKKVFYSFIDDKNHNKKLLVIRTKGTIAGQYRVYSEEGANKSGLAWPSAFKVQLQLPDNEVAQISDYYPRNSIDTKEYMSTLTYGFNGNVTGDDTGKIGGLIGANVSIGHTLKYVQPDFKTILESPTDKKVGWKVIFNNMVNQNWGPYDRDSWNPVYGNQLFMKTRNGSMKAADNFLDPNKASSLLSSGFSPDFATVITMDRKASKQQTNIDVIYERVRDDYQLHWTSTNWKGTNTKDKWTDRSSERYKIDWEKEEMTNGGSSGGSSGGAHIVMVDAYKPTKKGHHHHHHEAAAEAAAEAAAEAAAEAAAEAAAEAAAEAAAEAAAEAAAEAAAEAAAEAAAEEEEE

SEQ ID NO: 5 - protein, 310 aa, Artificial Sequence
  source: /note="Description of Artificial Sequence: Synthetic polypeptide"
ADSDINIKTGTTDIGSNTTVKTGDLVTYDKENGMGKKVFYSFIDDKNHNKKLLVIRTKGTIAGQYRVYSEEGANKSGLAWPSAFKVQLQLPDNEVAQISDYYPRNSIDTKEYMSTLTYGFNGNVTGDDTGKIGGLIGANVSIGATLKYVQPDFKTILESPTDKKVGWKVIFNNMVNQNWGPYDRDSWNPVYGNQLFMKTRNGSMKAADNFLDPNKASSLLSSGFSPDFATVITMDRKASKQQTNIDVIYERVRDDYQLHWTSTNWKGTNTKDKWTDRSSERYKIDWEKEEMTNGLSAENLYFQGHHHHHH

SEQ ID NO: 6 - protein, 267 aa, Unknown
  source: /note="Description of Unknown: OmpG sequence"
EERNDWHFNIGAMYEIENVEGYGEDMDGLAEPSVYFNAANGPWRIALAYKQEGPVDYSAGKRGTWFDRPELEVHYQFLENDDFSFGLTGGFRNYGYHYVDEPGKDTANMQRWKIAPDWDVKLTDDLRFNGWLSMYKFANDLNTTGYADTRVETETGLQYTFNETVALRVNYYLERGFNMDDSRNNGEFSTQEIRAYLPLTLGNHSVTPYTRIGLRAGHDFNRVGLFYGYDFQNGLSVSLEYAFEWQDHDEGDSDKFHYAGVGVNYSF

SEQ ID NO: 7 - protein, 355 aa, Artificial Sequence
  source: /note="Description of Artificial Sequence: Synthetic polypeptide"
EERNDWHFNIGAMYEIENVEGYGEDMDGLAEPSVYFNAANGPWRIALAYKQEGPVDYSAGKRGTWFDRPELEVHYQFLENDDFSFGLTGGFRNYGYHYVDEPGKDTANMQRWKIAPDWDVKLTDDLRFNGWLSMYKFANDLNTTGYADTRVETETGLQYTFNETVALRVNYYLERGFNMDDSRNNGEFSTQEIRAYLPLTLGNHSVTPYTRIGLRAGHDFNRVGLFYGYDFQNGLSVSLEYAFEWQDHDEGDSDKFHYAGVGVNYSFEKEKEKGSHHHHHHGSGGAHIVMVDAYKPTKEAAAEAAAEAAAEAAAEAAAEAAAEAAAEAAAEAAAEAAAEAAAEAAAEAAAEEEEE

SEQ ID NO: 8 - protein, 57 aa, Artificial Sequence
  source: /note="Description of Artificial Sequence: Synthetic polypeptide"
EAAAEAAAEAAAEAAAEAAAEAAAEAAAEAAAEAAAEAAAEAAAEAAAEAAAEEEEE

SEQ ID NO: 9 - protein, 229 aa, Artificial Sequence
  source: /note="Description of Artificial Sequence: Synthetic polypeptide"
QVQLVESGGALVQPGGSLRLSCAASGFPVNRYSMRWYRQAPGKEREWVAGMSSAGDRSSYEDSVKGRFTISRDDARNTVYLQMNSLKPEDTAVYYCNVNVGFEYWGQGTQVTVSSKGSGSGSDSATHIKFSKRDEDGKELAGATMELRDSSGKTISTWISDGQVKDFYLYPGKYTFVETAAPDGYEVATAITFTVNEQGQVTVNGKATKGDAHIENLYFQGHHHHHHHH

SEQ ID NO: 10 - protein, 373 aa, Artificial Sequence
  source: /note="Description of Artificial Sequence: Synthetic polypeptide"
SKGEELFTGVVPILVELDGDVNGHKFSVRGEGEGDATNGKLTLKFICTTGKLPVPWPTLVTTLGYGVQCFSRYPDHMKRHDFFKSAMPEGYVQERTISFKDGTYKTRAEVKFEGDTLVNRIELKGIDFKEDGNILGHKLEYNFNSHNVYITADKQKNGIKANFKIRHNVEDGSVQLADHYQQNTPIGDGPVLLPDNHYLSTQSKLSKDPNEKRDHMVLLEFVTAAGITHGMDELYKGSGGSGGSGGSGGSGGAMVDTLSGLSSEQGQSGDMTIEEDSATHIKFSKRDEDGKELAGATMELRDSSGKTISTWISDGQVKDFYLYPGKYTFVETAAPDGYEVATAITFTVNEQGQVTVNGKATKGDAHIHHHHHH

SEQ ID NO: 11 - protein, 14 aa, Artificial Sequence
  source: /note="Description of Artificial Sequence: Synthetic peptide"
AHIVMVDAYKPTKK

SEQ ID NO: 12 - protein, 10 aa, Artificial Sequence
  source: /note="Description of Artificial Sequence: Synthetic peptide"
GGSSGGSSGG

SEQ ID NO: 13 - protein, 8 aa, Artificial Sequence
  source: /note="Description of Artificial Sequence: Synthetic peptide"
EKEKEKGS

SEQ ID NO: 14 - protein, 4 aa, Artificial Sequence
  source: /note="Description of Artificial Sequence: Synthetic peptide"
GSGG

SEQ ID NO: 15 - protein, 6 aa, Artificial Sequence
  source: /note="Description of Artificial Sequence: Synthetic peptide"
GSGSGS

SEQ ID NO: 16 - protein, 293 aa, Staphylococcus aureus
ADSDINIKTGTTDIGSNTTVKTGDLVTYDKENGMHKKVFYSFIDDKNHNKKLLVIRTKGTIAGQYRVYSEEGANKSGLAWPSAFKVQLQLPDNEVAQISDYYPRNSIDTKEYMSTLTYGFNGNVTGDDTGKIGGLIGANVSIGHTLKYVQPDFKTILESPTDKKVGWKVIFNNMVNQNWGPYDRDSWNPVYGNQLFMKTRNGSMKAADNFLDPNKASSLLSSGFSPDFATVITMDRKASKQQTNIDVIYERVRDDYQLHWTSTNWKGTNTKDKWTDRSSERYKIDWEKEEMTN

SEQ ID NO: 17 - protein, 4 aa, Artificial Sequence
  source: /note="Description of Artificial Sequence: Synthetic peptide"
EPPP